European Patent Application EP 4 726 054 A1, published April 15, 2026. Title: 試料中の標的物質を検出する方法及びそのためのキット. Applicant: TOPPAN Holdings Inc. Application JP. The sequence listing filed with the application follows.

SEQUENCE LISTING (10 sequences)

SEQ ID NO: 1 - DNA, 51 bp, synthetic construct
  source 1..51: mol_type = other DNA
tttgtcactgttcctccttttgttttcctttctgtgagcaatttcacccaa

SEQ ID NO: 2 - DNA, 22 bp, synthetic construct
  source 1..22: mol_type = other DNA
gcatggttccaatttgggtgat

SEQ ID NO: 3 - DNA, 28 bp, synthetic construct
  source 1..28: mol_type = other DNA
cgcgccgaggaattgctcacagaaagga

SEQ ID NO: 4 - DNA, 35 bp, synthetic construct
  source 1..35: mol_type = other DNA
  misc_feature 1: note = modifyed with amino-C6-Alexa488
  misc_feature 5: note = modified with Black Hole Quencher (BHQ) -1
ttcttagccggttttccggctgagacctcggcgcg

SEQ ID NO: 5 - DNA, 24 bp, synthetic construct
  source 1..24: mol_type = other DNA
cgcgccgaggcgcagctcatgccc

SEQ ID NO: 6 - DNA, 101 bp, synthetic construct
  source 1..101: mol_type = other DNA
gccaggaacgtactggtgaaaacaccgcagcatgtcaagatcacagattttgggctggccaaactgctgggtgcggaagagaaagaataccatgcagaagg

SEQ ID NO: 7 - DNA, 31 bp, synthetic construct
  source 1..31: mol_type = other DNA
tctgcctcacctccaccgtgcarctcatcaa

SEQ ID NO: 8 - DNA, 28 bp, synthetic construct
  source 1..28: mol_type = other DNA
cgcgccgaggaattgctcacagaaagga

SEQ ID NO: 9 - DNA, 51 bp, synthetic construct; identical to SEQ ID NO: 1
  source 1..51: mol_type = other DNA

SEQ ID NO: 10 - DNA, 22 bp, synthetic construct
  source 1..22: mol_type = other DNA
gcatggttccaatttgggtgat